European Patent Application EP 4 620 474 A1, published September 24, 2025. Title: Method of treating a disorder with a C5a inhibitor. Applicant: Aptarion biotech AG. Application EP. The sequence listing filed with the application follows.

SEQUENCE LISTING (95 sequences)

SEQ ID NO: 1 - RNA, 44 nt, synthetic construct
  misc_feature 1..44: note = Synthetic
  misc_feature 1..44: note = L-nucleic acid
  source 1..44: mol_type = other RNA
gcctgatgtggtgttgaagggttgtggggtgtcgacgcacaggc

SEQ ID NO: 2 - RNA, 44 nt, synthetic construct
  misc_feature 1..44: note = Synthetic
  misc_feature 1..44: note = L-nucleic acid
  source 1..44: mol_type = other RNA
gcctgatgtggtgttgaggggttgtggggtgtcgacgcacaggc

SEQ ID NO: 3 - RNA, 44 nt, synthetic construct
  misc_feature 1..44: note = Synthetic
  misc_feature 1..44: note = L-nucleic acid
  source 1..44: mol_type = other RNA
gcctgatgtggtgttgaagggttgttgggtgtcgacgcacaggc

SEQ ID NO: 4 - RNA, 44 nt, synthetic construct
  misc_feature 1..44: note = Synthetic
  misc_feature 1..44: note = L-nucleic acid
  source 1..44: mol_type = other RNA
gcctgatgtggtggtgaagggttgttgggtgtcgacgcacaggc

SEQ ID NO: 5 - RNA, 44 nt, synthetic construct
  misc_feature 1..44: note = Synthetic
  misc_feature 1..44: note = L-nucleic acid
  source 1..44: mol_type = other RNA
gcctgatgtggtggtgaggggttgtggggtgtcgacgcacaggc

SEQ ID NO: 6 - RNA, 44 nt, synthetic construct
  misc_feature 1..44: note = Synthetic
  misc_feature 1..44: note = L-nucleic acid
  source 1..44: mol_type = other RNA
gcctgatgtggtggtgaggggatgtggggtgtcgacgcacaggc

SEQ ID NO: 7 - RNA, 44 nt, synthetic construct
  misc_feature 1..44: note = Synthetic
  misc_feature 1..44: note = L-nucleic acid
  source 1..44: mol_type = other RNA
gcctgatgtggtgttgaggggctgtggggtgtcgacgcacaggc

SEQ ID NO: 8 - RNA, 44 nt, synthetic construct; identical to SEQ ID NO: 4
  misc_feature 1..44: note = Synthetic
  misc_feature 1..44: note = L-nucleic acid
  misc_feature 9: note = Deoxyribonucleotide rather than ribonucleotide
  source 1..44: mol_type = other RNA

SEQ ID NO: 9 - RNA, 44 nt, synthetic construct; identical to SEQ ID NO: 4
  misc_feature 1..44: note = Synthetic
  misc_feature 1..44: note = L-nucleic acid
  misc_feature 16: note = Deoxyribonucleotide rather than ribonucleotide
  source 1..44: mol_type = other RNA

SEQ ID NO: 10 - RNA, 44 nt, synthetic construct; identical to SEQ ID NO: 4
  misc_feature 1..44: note = Synthetic
  misc_feature 1..44: note = L-nucleic acid
  misc_feature 17: note = Deoxyribonucleotide rather than ribonucleotide
  source 1..44: mol_type = other RNA

SEQ ID NO: 11 - RNA, 44 nt, synthetic construct; identical to SEQ ID NO: 4
  misc_feature 1..44: note = Synthetic
  misc_feature 1..44: note = L-nucleic acid
  misc_feature 30: note = Deoxyribonucleotide rather than ribonucleotide
  source 1..44: mol_type = other RNA

SEQ ID NO: 12 - RNA, 44 nt, synthetic construct; identical to SEQ ID NO: 4
  misc_feature 1..44: note = Synthetic
  misc_feature 1..44: note = L-nucleic acid
  misc_feature 32: note = Deoxyribonucleotide rather than ribonucleotide
  source 1..44: mol_type = other RNA

SEQ ID NO: 13 - RNA, 44 nt, synthetic construct; identical to SEQ ID NO: 4
  misc_feature 1..44: note = Synthetic
  misc_feature 1..44: note = L-nucleic acid
  misc_feature 40: note = Deoxyribonucleotide rather than ribonucleotide
  source 1..44: mol_type = other RNA

SEQ ID NO: 14 - RNA, 44 nt, synthetic construct; identical to SEQ ID NO: 4
  misc_feature 1..44: note = Synthetic
  misc_feature 1..44: note = L-nucleic acid
  misc_feature 9: note = Deoxyribonucleotide rather than ribonucleotide
  misc_feature 30: note = Deoxyribonucleotide rather than ribonucleotide
  source 1..44: mol_type = other RNA

SEQ ID NO: 15 - RNA, 44 nt, synthetic construct; identical to SEQ ID NO: 4
  misc_feature 1..44: note = Synthetic
  misc_feature 1..44: note = L-nucleic acid
  misc_feature 9: note = Deoxyribonucleotide rather than ribonucleotide
  misc_feature 32: note = Deoxyribonucleotide rather than ribonucleotide
  source 1..44: mol_type = other RNA

SEQ ID NO: 16 - RNA, 44 nt, synthetic construct; identical to SEQ ID NO: 4
  misc_feature 1..44: note = Synthetic
  misc_feature 1..44: note = L-nucleic acid
  misc_feature 9: note = Deoxyribonucleotide rather than ribonucleotide
  misc_feature 40: note = Deoxyribonucleotide rather than ribonucleotide
  source 1..44: mol_type = other RNA

SEQ ID NO: 17 - RNA, 44 nt, synthetic construct; identical to SEQ ID NO: 4
  misc_feature 1..44: note = Synthetic
  misc_feature 1..44: note = L-nucleic acid
  misc_feature 30: note = Deoxyribonucleotide rather than ribonucleotide
  misc_feature 32: note = Deoxyribonucleotide rather than ribonucleotide
  source 1..44: mol_type = other RNA

SEQ ID NO: 18 - RNA, 44 nt, synthetic construct; identical to SEQ ID NO: 4
  misc_feature 1..44: note = Synthetic
  misc_feature 1..44: note = L-nucleic acid
  misc_feature 30: note = Deoxyribonucleotide rather than ribonucleotide
  misc_feature 40: note = Deoxyribonucleotide rather than ribonucleotide
  source 1..44: mol_type = other RNA

SEQ ID NO: 19 - RNA, 44 nt, synthetic construct; identical to SEQ ID NO: 4
  misc_feature 1..44: note = Synthetic
  misc_feature 1..44: note = L-nucleic acid
  misc_feature 32: note = Deoxyribonucleotide rather than ribonucleotide
  misc_feature 40: note = Deoxyribonucleotide rather than ribonucleotide
  source 1..44: mol_type = other RNA

SEQ ID NO: 20 - RNA, 44 nt, synthetic construct; identical to SEQ ID NO: 4
  misc_feature 1..44: note = Synthetic
  misc_feature 1..44: note = L-nucleic acid
  misc_feature 9: note = Deoxyribonucleotide rather than ribonucleotide
  misc_feature 30: note = Deoxyribonucleotide rather than ribonucleotide
  misc_feature 32: note = Deoxyribonucleotide rather than ribonucleotide
  source 1..44: mol_type = other RNA

SEQ ID NO: 21 - RNA, 44 nt, synthetic construct; identical to SEQ ID NO: 4
  misc_feature 1..44: note = Synthetic
  misc_feature 1..44: note = L-nucleic acid
  misc_feature 9: note = Deoxyribonucleotide rather than ribonucleotide
  misc_feature 30: note = Deoxyribonucleotide rather than ribonucleotide
  misc_feature 40: note = Deoxyribonucleotide rather than ribonucleotide
  source 1..44: mol_type = other RNA

SEQ ID NO: 22 - RNA, 44 nt, synthetic construct; identical to SEQ ID NO: 4
  misc_feature 1..44: note = Synthetic
  misc_feature 1..44: note = L-nucleic acid
  misc_feature 9: note = Deoxyribonucleotide rather than ribonucleotide
  misc_feature 32: note = Deoxyribonucleotide rather than ribonucleotide
  misc_feature 40: note = Deoxyribonucleotide rather than ribonucleotide
  source 1..44: mol_type = other RNA

SEQ ID NO: 23 - RNA, 44 nt, synthetic construct; identical to SEQ ID NO: 4
  misc_feature 1..44: note = Synthetic
  misc_feature 1..44: note = L-nucleic acid
  misc_feature 30: note = Deoxyribonucleotide rather than ribonucleotide
  misc_feature 32: note = Deoxyribonucleotide rather than ribonucleotide
  misc_feature 40: note = Deoxyribonucleotide rather than ribonucleotide
  source 1..44: mol_type = other RNA

SEQ ID NO: 24 - RNA, 44 nt, synthetic construct; identical to SEQ ID NO: 4
  misc_feature 1..44: note = Synthetic
  misc_feature 1..44: note = L-nucleic acid
  misc_feature 9: note = Deoxyribonucleotide rather than ribonucleotide
  misc_feature 30: note = Deoxyribonucleotide rather than ribonucleotide
  misc_feature 32: note = Deoxyribonucleotide rather than ribonucleotide
  misc_feature 40: note = Deoxyribonucleotide rather than ribonucleotide
  source 1..44: mol_type = other RNA

SEQ ID NO: 25 - RNA, 44 nt, synthetic construct; identical to SEQ ID NO: 4
  misc_feature 1..44: note = Synthetic
  misc_feature 1..44: note = L-nucleic acid
  misc_feature 9: note = Deoxyribonucleotide rather than ribonucleotide
  misc_feature 16: note = Deoxyribonucleotide rather than ribonucleotide
  misc_feature 30: note = Deoxyribonucleotide rather than ribonucleotide
  misc_feature 32: note = Deoxyribonucleotide rather than ribonucleotide
  misc_feature 40: note = Deoxyribonucleotide rather than ribonucleotide
  source 1..44: mol_type = other RNA

SEQ ID NO: 26 - RNA, 44 nt, synthetic construct; identical to SEQ ID NO: 4
  misc_feature 1..44: note = Synthetic
  misc_feature 1..44: note = L-nucleic acid
  misc_feature 9: note = Deoxyribonucleotide rather than ribonucleotide
  misc_feature 17: note = Deoxyribonucleotide rather than ribonucleotide
  misc_feature 30: note = Deoxyribonucleotide rather than ribonucleotide
  misc_feature 32: note = Deoxyribonucleotide rather than ribonucleotide
  misc_feature 40: note = Deoxyribonucleotide rather than ribonucleotide
  source 1..44: mol_type = other RNA

SEQ ID NO: 27 - RNA, 44 nt, synthetic construct; identical to SEQ ID NO: 4
  misc_feature 1..44: note = Synthetic
  misc_feature 1..44: note = L-nucleic acid
  misc_feature 9: note = Deoxyribonucleotide rather than ribonucleotide
  misc_feature 16: note = Deoxyribonucleotide rather than ribonucleotide
  misc_feature 17: note = Deoxyribonucleotide rather than ribonucleotide
  misc_feature 30: note = Deoxyribonucleotide rather than ribonucleotide
  misc_feature 32: note = Deoxyribonucleotide rather than ribonucleotide
  misc_feature 40: note = Deoxyribonucleotide rather than ribonucleotide
  source 1..44: mol_type = other RNA

SEQ ID NO: 28 - RNA, 43 nt, synthetic construct
  misc_feature 1..43: note = Synthetic
  misc_feature 1..43: note = L-nucleic acid
  misc_feature 8: note = Deoxyribonucleotide rather than ribonucleotide
  misc_feature 15: note = Deoxyribonucleotide rather than ribonucleotide
  misc_feature 16: note = Deoxyribonucleotide rather than ribonucleotide
  misc_feature 29: note = Deoxyribonucleotide rather than ribonucleotide
  misc_feature 31: note = Deoxyribonucleotide rather than ribonucleotide
  misc_feature 39: note = Deoxyribonucleotide rather than ribonucleotide
  source 1..43: mol_type = other RNA
cctgatgtggtggtgaagggttgttgggtgtcgacgcacaggc

SEQ ID NO: 29 - RNA, 42 nt, synthetic construct
  misc_feature 1..42: note = Synthetic
  misc_feature 1..42: note = L-nucleic acid
  misc_feature 7: note = Deoxyribonucleotide rather than ribonucleotide
  misc_feature 14: note = Deoxyribonucleotide rather than ribonucleotide
  misc_feature 15: note = Deoxyribonucleotide rather than ribonucleotide
  misc_feature 28: note = Deoxyribonucleotide rather than ribonucleotide
  misc_feature 30: note = Deoxyribonucleotide rather than ribonucleotide
  misc_feature 38: note = Deoxyribonucleotide rather than ribonucleotide
  source 1..42: mol_type = other RNA
ctgatgtggtggtgaagggttgttgggtgtcgacgcacaggc

SEQ ID NO: 30 - RNA, 41 nt, synthetic construct
  misc_feature 1..41: note = Synthetic
  misc_feature 1..41: note = L-nucleic acid
  misc_feature 6: note = Deoxyribonucleotide rather than ribonucleotide
  misc_feature 13: note = Deoxyribonucleotide rather than ribonucleotide
  misc_feature 14: note = Deoxyribonucleotide rather than ribonucleotide
  misc_feature 27: note = Deoxyribonucleotide rather than ribonucleotide
  misc_feature 29: note = Deoxyribonucleotide rather than ribonucleotide
  misc_feature 37: note = Deoxyribonucleotide rather than ribonucleotide
  source 1..41: mol_type = other RNA
tgatgtggtggtgaagggttgttgggtgtcgacgcacaggc

SEQ ID NO: 31 - RNA, 40 nt, synthetic construct
  misc_feature 1..40: note = Synthetic
  misc_feature 1..40: note = L-nucleic acid
  misc_feature 5: note = Deoxyribonucleotide rather than ribonucleotide
  misc_feature 12: note = Deoxyribonucleotide rather than ribonucleotide
  misc_feature 13: note = Deoxyribonucleotide rather than ribonucleotide
  misc_feature 26: note = Deoxyribonucleotide rather than ribonucleotide
  misc_feature 28: note = Deoxyribonucleotide rather than ribonucleotide
  misc_feature 36: note = Deoxyribonucleotide rather than ribonucleotide
  source 1..40: mol_type = other RNA
gatgtggtggtgaagggttgttgggtgtcgacgcacaggc

SEQ ID NO: 32 - RNA, 42 nt, synthetic construct
  misc_feature 1..42: note = Synthetic
  misc_feature 1..42: note = L-nucleic acid
  misc_feature 8: note = Deoxyribonucleotide rather than ribonucleotide
  misc_feature 15: note = Deoxyribonucleotide rather than ribonucleotide
  misc_feature 16: note = Deoxyribonucleotide rather than ribonucleotide
  misc_feature 29: note = Deoxyribonucleotide rather than ribonucleotide
  misc_feature 31: note = Deoxyribonucleotide rather than ribonucleotide
  misc_feature 39: note = Deoxyribonucleotide rather than ribonucleotide
  source 1..42: mol_type = other RNA
gctgatgtggtggtgaagggttgttgggtgtcgacgcacagc

SEQ ID NO: 33 - RNA, 40 nt, synthetic construct
  misc_feature 1..40: note = Synthetic
  misc_feature 1..40: note = L-nucleic acid
  misc_feature 7: note = Deoxyribonucleotide rather than ribonucleotide
  misc_feature 14: note = Deoxyribonucleotide rather than ribonucleotide
  misc_feature 15: note = Deoxyribonucleotide rather than ribonucleotide
  misc_feature 28: note = Deoxyribonucleotide rather than ribonucleotide
  misc_feature 30: note = Deoxyribonucleotide rather than ribonucleotide
  misc_feature 38: note = Deoxyribonucleotide rather than ribonucleotide
  source 1..40: mol_type = other RNA
gtgatgtggtggtgaagggttgttgggtgtcgacgcacac

SEQ ID NO: 34 - RNA, 38 nt, synthetic construct
  misc_feature 1..38: note = Synthetic
  misc_feature 1..38: note = L-nucleic acid
  misc_feature 6: note = Deoxyribonucleotide rather than ribonucleotide
  misc_feature 13: note = Deoxyribonucleotide rather than ribonucleotide
  misc_feature 14: note = Deoxyribonucleotide rather than ribonucleotide
  misc_feature 27: note = Deoxyribonucleotide rather than ribonucleotide
  misc_feature 29: note = Deoxyribonucleotide rather than ribonucleotide
  misc_feature 37: note = Deoxyribonucleotide rather than ribonucleotide
  source 1..38: mol_type = other RNA
tgatgtggtggtgaagggttgttgggtgtcgacgcaca

SEQ ID NO: 35 - RNA, 42 nt, synthetic construct
  misc_feature 1..42: note = Synthetic
  misc_feature 1..42: note = L-nucleic acid
  misc_feature 8: note = Deoxyribonucleotide rather than ribonucleotide
  misc_feature 15: note = Deoxyribonucleotide rather than ribonucleotide
  misc_feature 16: note = Deoxyribonucleotide rather than ribonucleotide
  misc_feature 29: note = Deoxyribonucleotide rather than ribonucleotide
  misc_feature 31: note = Deoxyribonucleotide rather than ribonucleotide
  misc_feature 39: note = Deoxyribonucleotide rather than ribonucleotide
  source 1..42: mol_type = other RNA
gccgatgtggtggtgaagggttgttgggtgtcgacgcacggc

SEQ ID NO: 36 - RNA, 42 nt, synthetic construct
  misc_feature 1..42: note = Synthetic
  misc_feature 1..42: note = L-nucleic acid
  misc_feature 8: note = Deoxyribonucleotide rather than ribonucleotide
  misc_feature 15: note = Deoxyribonucleotide rather than ribonucleotide
  misc_feature 16: note = Deoxyribonucleotide rather than ribonucleotide
  misc_feature 29: note = Deoxyribonucleotide rather than ribonucleotide
  misc_feature 31: note = Deoxyribonucleotide rather than ribonucleotide
  misc_feature 39: note = Deoxyribonucleotide rather than ribonucleotide
  source 1..42: mol_type = other RNA
ggcgatgtggtggtgaagggttgttgggtgtcgacgcacgcc

SEQ ID NO: 37 - RNA, 40 nt, synthetic construct
  misc_feature 1..40: note = Synthetic
  misc_feature 1..40: note = L-nucleic acid
  misc_feature 7: note = Deoxyribonucleotide rather than ribonucleotide
  misc_feature 14: note = Deoxyribonucleotide rather than ribonucleotide
  misc_feature 15: note = Deoxyribonucleotide rather than ribonucleotide
  misc_feature 28: note = Deoxyribonucleotide rather than ribonucleotide
  misc_feature 30: note = Deoxyribonucleotide rather than ribonucleotide
  misc_feature 38: note = Deoxyribonucleotide rather than ribonucleotide
  source 1..40: mol_type = other RNA
gcgatgtggtggtgaagggttgttgggtgtcgacgcacgc

SEQ ID NO: 38 - RNA, 41 nt, synthetic construct
  misc_feature 1..41: note = Synthetic
  misc_feature 1..41: note = L-nucleic acid
  misc_feature 7: note = Deoxyribonucleotide rather than ribonucleotide
  misc_feature 14: note = Deoxyribonucleotide rather than ribonucleotide
  misc_feature 15: note = Deoxyribonucleotide rather than ribonucleotide
  misc_feature 28: note = Deoxyribonucleotide rather than ribonucleotide
  misc_feature 30: note = Deoxyribonucleotide rather than ribonucleotide
  misc_feature 38: note = Deoxyribonucleotide rather than ribonucleotide
  source 1..41: mol_type = other RNA
ctgatgtggtggtgaagggttgttgggtgtcgacgcacagc

SEQ ID NO: 39 - RNA, 40 nt, synthetic construct
  misc_feature 1..40: note = Synthetic
  misc_feature 1..40: note = L-nucleic acid
  misc_feature 6: note = Deoxyribonucleotide rather than ribonucleotide
  misc_feature 13: note = Deoxyribonucleotide rather than ribonucleotide
  misc_feature 14: note = Deoxyribonucleotide rather than ribonucleotide
  misc_feature 27: note = Deoxyribonucleotide rather than ribonucleotide
  misc_feature 29: note = Deoxyribonucleotide rather than ribonucleotide
  misc_feature 37: note = Deoxyribonucleotide rather than ribonucleotide
  source 1..40: mol_type = other RNA
tgatgtggtggtgaagggttgttgggtgtcgacgcacagc

SEQ ID NO: 40 - RNA, 40 nt, synthetic construct
  misc_feature 1..40: note = Synthetic
  misc_feature 1..40: note = L-nucleic acid
  misc_feature 6: note = Deoxyribonucleotide rather than ribonucleotide
  misc_feature 13: note = Deoxyribonucleotide rather than ribonucleotide
  misc_feature 14: note = Deoxyribonucleotide rather than ribonucleotide
  misc_feature 27: note = Deoxyribonucleotide rather than ribonucleotide
  misc_feature 29: note = Deoxyribonucleotide rather than ribonucleotide
  misc_feature 37: note = Deoxyribonucleotide rather than ribonucleotide
  source 1..40: mol_type = other RNA
cgatgtggtggtgaagggttgttgggtgtcgacgcacagc

SEQ ID NO: 41 - RNA, 39 nt, synthetic construct
  misc_feature 1..39: note = Synthetic
  misc_feature 1..39: note = L-nucleic acid
  misc_feature 5: note = Deoxyribonucleotide rather than ribonucleotide
  misc_feature 12: note = Deoxyribonucleotide rather than ribonucleotide
  misc_feature 13: note = Deoxyribonucleotide rather than ribonucleotide
  misc_feature 26: note = Deoxyribonucleotide rather than ribonucleotide
  misc_feature 28: note = Deoxyribonucleotide rather than ribonucleotide
  misc_feature 36: note = Deoxyribonucleotide rather than ribonucleotide
  source 1..39: mol_type = other RNA
gatgtggtggtgaagggttgttgggtgtcgacgcacagc

SEQ ID NO: 42 - RNA, 41 nt, synthetic construct
  misc_feature 1..41: note = Synthetic
  misc_feature 1..41: note = L-nucleic acid
  misc_feature 8: note = Deoxyribonucleotide rather than ribonucleotide
  misc_feature 15: note = Deoxyribonucleotide rather than ribonucleotide
  misc_feature 16: note = Deoxyribonucleotide rather than ribonucleotide
  misc_feature 29: note = Deoxyribonucleotide rather than ribonucleotide
  misc_feature 31: note = Deoxyribonucleotide rather than ribonucleotide
  misc_feature 39: note = Deoxyribonucleotide rather than ribonucleotide
  source 1..41: mol_type = other RNA
gctgatgtggtggtgaagggttgttgggtgtcgacgcacac

SEQ ID NO: 43 - RNA, 40 nt, synthetic construct
  misc_feature 1..40: note = Synthetic
  misc_feature 1..40: note = L-nucleic acid
  misc_feature 8: note = Deoxyribonucleotide rather than ribonucleotide
  misc_feature 15: note = Deoxyribonucleotide rather than ribonucleotide
  misc_feature 16: note = Deoxyribonucleotide rather than ribonucleotide
  misc_feature 29: note = Deoxyribonucleotide rather than ribonucleotide
  misc_feature 31: note = Deoxyribonucleotide rather than ribonucleotide
  misc_feature 39: note = Deoxyribonucleotide rather than ribonucleotide
  source 1..40: mol_type = other RNA
gctgatgtggtggtgaagggttgttgggtgtcgacgcacc

SEQ ID NO: 44 - RNA, 40 nt, synthetic construct
  misc_feature 1..40: note = Synthetic
  misc_feature 1..40: note = L-nucleic acid
  misc_feature 8: note = Deoxyribonucleotide rather than ribonucleotide
  misc_feature 15: note = Deoxyribonucleotide rather than ribonucleotide
  misc_feature 16: note = Deoxyribonucleotide rather than ribonucleotide
  misc_feature 29: note = Deoxyribonucleotide rather than ribonucleotide
  misc_feature 31: note = Deoxyribonucleotide rather than ribonucleotide
  misc_feature 39: note = Deoxyribonucleotide rather than ribonucleotide
  source 1..40: mol_type = other RNA
gctgatgtggtggtgaagggttgttgggtgtcgacgcaca

SEQ ID NO: 45 - RNA, 39 nt, synthetic construct
  misc_feature 1..39: note = Synthetic
  misc_feature 1..39: note = L-nucleic acid
  misc_feature 6: note = Deoxyribonucleotide rather than ribonucleotide
  misc_feature 13: note = Deoxyribonucleotide rather than ribonucleotide
  misc_feature 14: note = Deoxyribonucleotide rather than ribonucleotide
  misc_feature 27: note = Deoxyribonucleotide rather than ribonucleotide
  misc_feature 29: note = Deoxyribonucleotide rather than ribonucleotide
  misc_feature 37: note = Deoxyribonucleotide rather than ribonucleotide
  source 1..39: mol_type = other RNA
cgatgtggtggtgaagggttgttgggtgtcgacgcacgc

SEQ ID NO: 46 - RNA, 38 nt, synthetic construct
  misc_feature 1..38: note = Synthetic
  misc_feature 1..38: note = L-nucleic acid
  misc_feature 5: note = Deoxyribonucleotide rather than ribonucleotide
  misc_feature 12: note = Deoxyribonucleotide rather than ribonucleotide
  misc_feature 13: note = Deoxyribonucleotide rather than ribonucleotide
  misc_feature 26: note = Deoxyribonucleotide rather than ribonucleotide
  misc_feature 28: note = Deoxyribonucleotide rather than ribonucleotide
  misc_feature 36: note = Deoxyribonucleotide rather than ribonucleotide
  source 1..38: mol_type = other RNA
gatgtggtggtgaagggttgttgggtgtcgacgcacgc

SEQ ID NO: 47 - RNA, 39 nt, synthetic construct
  misc_feature 1..39: note = Synthetic
  misc_feature 1..39: note = L-nucleic acid
  misc_feature 7: note = Deoxyribonucleotide rather than ribonucleotide
  misc_feature 14: note = Deoxyribonucleotide rather than ribonucleotide
  misc_feature 15: note = Deoxyribonucleotide rather than ribonucleotide
  misc_feature 28: note = Deoxyribonucleotide rather than ribonucleotide
  misc_feature 30: note = Deoxyribonucleotide rather than ribonucleotide
  misc_feature 38: note = Deoxyribonucleotide rather than ribonucleotide
  source 1..39: mol_type = other RNA
gcgatgtggtggtgaagggttgttgggtgtcgacgcacc

SEQ ID NO: 48 - RNA, 38 nt, synthetic construct
  misc_feature 1..38: note = Synthetic
  misc_feature 1..38: note = L-nucleic acid
  misc_feature 7: note = Deoxyribonucleotide rather than ribonucleotide
  misc_feature 14: note = Deoxyribonucleotide rather than ribonucleotide
  misc_feature 15: note = Deoxyribonucleotide rather than ribonucleotide
  misc_feature 28: note = Deoxyribonucleotide rather than ribonucleotide
  misc_feature 30: note = Deoxyribonucleotide rather than ribonucleotide
  misc_feature 38: note = Deoxyribonucleotide rather than ribonucleotide
  source 1..38: mol_type = other RNA
gcgatgtggtggtgaagggttgttgggtgtcgacgcac

SEQ ID NO: 49 - RNA, 38 nt, synthetic construct
  misc_feature 1..38: note = Synthetic
  misc_feature 1..38: note = L-nucleic acid
  misc_feature 6: note = Deoxyribonucleotide rather than ribonucleotide
  misc_feature 13: note = Deoxyribonucleotide rather than ribonucleotide
  misc_feature 14: note = Deoxyribonucleotide rather than ribonucleotide
  misc_feature 27: note = Deoxyribonucleotide rather than ribonucleotide
  misc_feature 29: note = Deoxyribonucleotide rather than ribonucleotide
  misc_feature 37: note = Deoxyribonucleotide rather than ribonucleotide
  source 1..38: mol_type = other RNA
ggatgtggtggtgaagggttgttgggtgtcgacgcacc

SEQ ID NO: 50 - protein, 74 aa, Homo sapiens
TLQKKIEEIAAKYKHSVVKKCCYDGACVNNDETCEQRAARISLGPRCIKAFTECCVVASQLRANISHKDMQLGR

SEQ ID NO: 51 - protein, 77 aa, Rattus norvegicus
DLQLLHQKVEEQAAKYKHRVPKKCCYDGARENKYETCEQRVARVTIGPHCIRAFNECCTIADKIRKESHHKGMLLGR

SEQ ID NO: 52 - protein, 77 aa, Mus musculus
NLHLLRQKIEEQAAKYKHSVPKKCCYDGARVNFYETCEERVARVTIGPLCIRAFNECCTIANKIRKESPHKPVQLGR

SEQ ID NO: 53 - protein, 999 aa, Homo sapiens
TLQKKIEEIAAKYKHSVVKKCCYDGACVNNDETCEQRAARISLGPRCIKAFTECCVVASQLRANISHKDMQLGRLHMKTLLPVSKPEIRSYFPESWLWEVHLVPRRKQLQFALPDSLTTWEIQGIGISNTGICVADTVKAKVFKDVFLEMNIPYSVVRGEQIQLKGTVYNYRTSGMQFCVKMSAVEGICTSESPVIDHQGTKSSKCVRQKVEGSSSHLVTFTVLPLEIGLHNINFSLETWFGKEILVKTLRVVPEGVKRESYSGVTLDPRGIYGTISRRKEFPYRIPLDLVPKTEIKRILSVKGLLVGEILSAVLSQEGINILTHLPKGSAEAELMSVVPVFYVFHYLETGNHWNIFHSDPLIEKQKLKKKLKEGMLSIMSYRNADYSYSVWKGGSASTWLTAFALRVLGQVNKYVEQNQNSICNSLLWLVENYQLDNGSFKENSQYQPIKLQGTLPVEARENSLYLTAFTVIGIRKAFDICPLVKIDTALIKADNFLLENTLPAQSTFTLAISAYALSLGDKTHPQFRSIVSALKREALVKGNPPIYRFWKDNLQHKDSSVPNTGTARMVETTAYALLTSLNLKDINYVNPVIKWLSEEQRYGGGFYSTQDTINAIEGLTEYSLLVKQLRLSMDIDVSYKHKGALHNYKMTDKNFLGRPVEVLLNDDLIVSTGFGSGLATVHVTTVVHKTSTSEEVCSFYLKIDTQDIEASHYRGYGNSDYKRIVACASYKPSREESSSGSSHAVMDISLPTGISANEEDLKALVEGVDQLFTDYQIKDGHVILQLNSIPSSDFLCVRFRIFELFEVGFLSPATFTVYEYHRPDKQCTMFYSTSNIKIQKVCEGAACKCVEADCGQMQEELDLTISAETRKQTACKPEIAYAYKVSITSITVENVFVKYKATLLDIYKTGEAVAEKDSEITFIKKVTCTNAELVKGRQYLIMGKEALQIKYNFSFRYIYPLDSLTWIEYWPRDTTCSSCQAFLANLDEFAEDIFLNGC

SEQ ID NO: 54 - protein, 74 aa, Macaca mulatta
MLQEKIEEIAAKYKHLVVKKCCYDGVRINHDETCEQRAARISVGPRCVKAFTECCVVASQLRANNSHKDLQLGR

SEQ ID NO: 55 - RNA, 40 nt, synthetic construct; identical to SEQ ID NO: 37
  misc_feature 1..40: note = Synthetic
  source 1..40: mol_type = other RNA

SEQ ID NO: 56 - RNA, 40 nt, synthetic construct; identical to SEQ ID NO: 37
  misc_feature 1..40: note = Synthetic
  misc_feature 1..40: note = L-nucleic acid
  misc_feature 7: note = Deoxyribonucleotide rather than ribonucleotide
  source 1..40: mol_type = other RNA

SEQ ID NO: 57 - RNA, 40 nt, synthetic construct; identical to SEQ ID NO: 37
  misc_feature 1..40: note = Synthetic
  misc_feature 1..40: note = L-nucleic acid
  misc_feature 7: note = Deoxyribonucleotide rather than ribonucleotide
  misc_feature 28: note = Deoxyribonucleotide rather than ribonucleotide
  source 1..40: mol_type = other RNA

SEQ ID NO: 58 - RNA, 40 nt, synthetic construct; identical to SEQ ID NO: 37
  misc_feature 1..40: note = Synthetic
  misc_feature 1..40: note = L-nucleic acid
  misc_feature 7: note = Deoxyribonucleotide rather than ribonucleotide
  misc_feature 28: note = Deoxyribonucleotide rather than ribonucleotide
  misc_feature 30: note = Deoxyribonucleotide rather than ribonucleotide
  source 1..40: mol_type = other RNA

SEQ ID NO: 59 - RNA, 40 nt, synthetic construct; identical to SEQ ID NO: 37
  misc_feature 1..40: note = Synthetic
  misc_feature 1..40: note = L-nucleic acid
  misc_feature 7: note = Deoxyribonucleotide rather than ribonucleotide
  misc_feature 28: note = Deoxyribonucleotide rather than ribonucleotide
  misc_feature 38: note = Deoxyribonucleotide rather than ribonucleotide
  source 1..40: mol_type = other RNA

SEQ ID NO: 60 - RNA, 40 nt, synthetic construct; identical to SEQ ID NO: 37
  misc_feature 1..40: note = Synthetic
  misc_feature 1..40: note = L-nucleic acid
  misc_feature 7: note = Deoxyribonucleotide rather than ribonucleotide
  misc_feature 28: note = Deoxyribonucleotide rather than ribonucleotide
  misc_feature 30: note = Deoxyribonucleotide rather than ribonucleotide
  misc_feature 38: note = Deoxyribonucleotide rather than ribonucleotide
  source 1..40: mol_type = other RNA

SEQ ID NO: 61 - RNA, 34 nt, synthetic construct
  misc_feature 1..34: note = Synthetic
  misc_feature 1..34: note = L-nucleic acid
  misc_feature 4: note = n is U or dU
  misc_feature 11: note = n is G or dG
  misc_feature 12: note = n is A or dA
  misc_feature 25: note = n is U or dU
  misc_feature 27: note = n is U or dU
  source 1..34: mol_type = other RNA
atgnggtgktnnrggghtgtkgggngncgacgca

SEQ ID NO: 62 - RNA, 34 nt, synthetic construct
  misc_feature 1..34: note = Synthetic
  misc_feature 1..34: note = L-nucleic acid
  misc_feature 4: note = n is U or dU
  misc_feature 11: note = n is G or dG
  misc_feature 12: note = n is A or dA
  misc_feature 25: note = n is U or dU
  misc_feature 27: note = n is U or dU
  source 1..34: mol_type = other RNA
atgnggtgttnnagggttgtggggngncgacgca

SEQ ID NO: 63 - RNA, 34 nt, synthetic construct
  misc_feature 1..34: note = Synthetic
  misc_feature 1..34: note = L-nucleic acid
  misc_feature 4: note = n is U or dU
  misc_feature 11: note = n is G or dG
  misc_feature 12: note = n is A or dA
  misc_feature 25: note = n is U or dU
  misc_feature 27: note = n is U or dU
  source 1..34: mol_type = other RNA
atgnggtgttnnggggttgtggggngncgacgca

SEQ ID NO: 64 - RNA, 34 nt, synthetic construct
  misc_feature 1..34: note = Synthetic
  misc_feature 1..34: note = L-nucleic acid
  misc_feature 4: note = n is U or dU
  misc_feature 11: note = n is G or dG
  misc_feature 12: note = n is A or dA
  misc_feature 25: note = n is U or dU
  misc_feature 27: note = n is U or dU
  source 1..34: mol_type = other RNA
atgnggtgttnnagggttgttgggngncgacgca

SEQ ID NO: 65 - RNA, 34 nt, synthetic construct
  misc_feature 1..34: note = Synthetic
  misc_feature 1..34: note = L-nucleic acid
  misc_feature 4: note = n is U or dU
  misc_feature 11: note = n is G or dG
  misc_feature 12: note = n is A or dA
  misc_feature 25: note = n is U or dU
  misc_feature 27: note = n is U or dU
  source 1..34: mol_type = other RNA
atgnggtggtnnagggttgttgggngncgacgca

SEQ ID NO: 66 - RNA, 34 nt, synthetic construct
  misc_feature 1..34: note = Synthetic
  misc_feature 1..34: note = L-nucleic acid
  misc_feature 4: note = n is U or dU
  misc_feature 11: note = n is G or dG
  misc_feature 12: note = n is A or dA
  misc_feature 25: note = n is U or dU
  misc_feature 27: note = n is U or dU
  source 1..34: mol_type = other RNA
atgnggtggtnnggggttgtggggngncgacgca

SEQ ID NO: 67 - RNA, 34 nt, synthetic construct
  misc_feature 1..34: note = Synthetic
  misc_feature 1..34: note = L-nucleic acid
  misc_feature 4: note = n is U or dU
  misc_feature 11: note = n is G or dG
  misc_feature 12: note = n is A or dA
  misc_feature 25: note = n is U or dU
  misc_feature 27: note = n is U or dU
  source 1..34: mol_type = other RNA
atgnggtggtnnggggatgtggggngncgacgca

SEQ ID NO: 68 - RNA, 34 nt, synthetic construct
  misc_feature 1..34: note = Synthetic
  misc_feature 1..34: note = L-nucleic acid
  misc_feature 4: note = n is U or dU
  misc_feature 11: note = n is G or dG
  misc_feature 12: note = n is A or dA
  misc_feature 25: note = n is U or dU
  misc_feature 27: note = n is U or dU
  source 1..34: mol_type = other RNA
atgnggtgttnnggggctgtggggngncgacgca

SEQ ID NO: 69 - RNA, 34 nt, synthetic construct
  misc_feature 1..34: note = Synthetic
  misc_feature 1..34: note = L-nucleic acid
  source 1..34: mol_type = other RNA
atgtggtgktgarggghtgtkgggtgtcgacgca

SEQ ID NO: 70 - RNA, 34 nt, synthetic construct
  misc_feature 1..34: note = Synthetic
  misc_feature 1..34: note = L-nucleic acid
  source 1..34: mol_type = other RNA
atgtggtgttgaagggttgttgggtgtcgacgca

SEQ ID NO: 71 - RNA, 34 nt, synthetic construct
  misc_feature 1..34: note = Synthetic
  misc_feature 1..34: note = L-nucleic acid
  source 1..34: mol_type = other RNA
atgtggtggtgaagggttgttgggtgtcgacgca

SEQ ID NO: 72 - RNA, 34 nt, synthetic construct
  misc_feature 1..34: note = Synthetic
  misc_feature 1..34: note = L-nucleic acid
  source 1..34: mol_type = other RNA
atgtggtggtgaggggttgtggggtgtcgacgca

SEQ ID NO: 73 - RNA, 34 nt, synthetic construct; identical to SEQ ID NO: 71
  misc_feature 1..34: note = Synthetic
  misc_feature 1..34: note = L-nucleic acid
  misc_feature 4: note = Deoxyribonucleotide rather than ribonucleotide
  source 1..34: mol_type = other RNA

SEQ ID NO: 74 - RNA, 34 nt, synthetic construct; identical to SEQ ID NO: 71
  misc_feature 1..34: note = Synthetic
  misc_feature 1..34: note = L-nucleic acid
  misc_feature 11: note = Deoxyribonucleotide rather than ribonucleotide
  source 1..34: mol_type = other RNA

SEQ ID NO: 75 - RNA, 34 nt, synthetic construct; identical to SEQ ID NO: 71
  misc_feature 1..34: note = Synthetic
  misc_feature 1..34: note = L-nucleic acid
  misc_feature 12: note = Deoxyribonucleotide rather than ribonucleotide
  source 1..34: mol_type = other RNA

SEQ ID NO: 76 - RNA, 34 nt, synthetic construct; identical to SEQ ID NO: 71
  misc_feature 1..34: note = Synthetic
  misc_feature 1..34: note = L-nucleic acid
  misc_feature 25: note = Deoxyribonucleotide rather than ribonucleotide
  source 1..34: mol_type = other RNA

SEQ ID NO: 77 - RNA, 34 nt, synthetic construct; identical to SEQ ID NO: 71
  misc_feature 1..34: note = Synthetic
  misc_feature 1..34: note = L-nucleic acid
  misc_feature 27: note = Deoxyribonucleotide rather than ribonucleotide
  source 1..34: mol_type = other RNA

SEQ ID NO: 78 - RNA, 34 nt, synthetic construct; identical to SEQ ID NO: 71
  misc_feature 1..34: note = Synthetic
  misc_feature 1..34: note = L-nucleic acid
  misc_feature 4: note = Deoxyribonucleotide rather than ribonucleotide
  misc_feature 25: note = Deoxyribonucleotide rather than ribonucleotide
  source 1..34: mol_type = other RNA

SEQ ID NO: 79 - RNA, 34 nt, synthetic construct; identical to SEQ ID NO: 71
  misc_feature 1..34: note = Synthetic
  misc_feature 1..34: note = L-nucleic acid
  misc_feature 4: note = Deoxyribonucleotide rather than ribonucleotide
  misc_feature 27: note = Deoxyribonucleotide rather than ribonucleotide
  source 1..34: mol_type = other RNA

SEQ ID NO: 80 - RNA, 34 nt, synthetic construct; identical to SEQ ID NO: 71
  misc_feature 1..34: note = Synthetic
  misc_feature 1..34: note = L-nucleic acid
  misc_feature 25: note = Deoxyribonucleotide rather than ribonucleotide
  misc_feature 27: note = Deoxyribonucleotide rather than ribonucleotide
  source 1..34: mol_type = other RNA

SEQ ID NO: 81 - RNA, 34 nt, synthetic construct; identical to SEQ ID NO: 71
  misc_feature 1..34: note = Synthetic
  misc_feature 1..34: note = L-nucleic acid
  misc_feature 4: note = Deoxyribonucleotide rather than ribonucleotide
  misc_feature 25: note = Deoxyribonucleotide rather than ribonucleotide
  misc_feature 27: note = Deoxyribonucleotide rather than ribonucleotide
  source 1..34: mol_type = other RNA

SEQ ID NO: 82 - RNA, 34 nt, synthetic construct; identical to SEQ ID NO: 71
  misc_feature 1..34: note = Synthetic
  misc_feature 1..34: note = L-nucleic acid
  misc_feature 4: note = Deoxyribonucleotide rather than ribonucleotide
  misc_feature 11: note = Deoxyribonucleotide rather than ribonucleotide
  misc_feature 25: note = Deoxyribonucleotide rather than ribonucleotide
  misc_feature 27: note = Deoxyribonucleotide rather than ribonucleotide
  source 1..34: mol_type = other RNA

SEQ ID NO: 83 - RNA, 34 nt, synthetic construct; identical to SEQ ID NO: 71
  misc_feature 1..34: note = Synthetic
  misc_feature 1..34: note = L-nucleic acid
  misc_feature 4: note = Deoxyribonucleotide rather than ribonucleotide
  misc_feature 12: note = Deoxyribonucleotide rather than ribonucleotide
  misc_feature 25: note = Deoxyribonucleotide rather than ribonucleotide
  misc_feature 27: note = Deoxyribonucleotide rather than ribonucleotide
  source 1..34: mol_type = other RNA

SEQ ID NO: 84 - RNA, 34 nt, synthetic construct; identical to SEQ ID NO: 71
  misc_feature 1..34: note = Synthetic
  misc_feature 1..34: note = L-nucleic acid
  misc_feature 4: note = Deoxyribonucleotide rather than ribonucleotide
  misc_feature 11: note = Deoxyribonucleotide rather than ribonucleotide
  misc_feature 12: note = Deoxyribonucleotide rather than ribonucleotide
  misc_feature 25: note = Deoxyribonucleotide rather than ribonucleotide
  misc_feature 27: note = Deoxyribonucleotide rather than ribonucleotide
  source 1..34: mol_type = other RNA

SEQ ID NO: 85 - RNA, 44 nt, synthetic construct; identical to SEQ ID NO: 7
  misc_feature 1..44: note = Synthetic
  misc_feature 1..44: note = D-nucleic acid
  source 1..44: mol_type = other RNA

SEQ ID NO: 86 - RNA, 44 nt, synthetic construct; identical to SEQ ID NO: 2
  misc_feature 1..44: note = Synthetic
  misc_feature 1..44: note = D-nucleic acid
  source 1..44: mol_type = other RNA

SEQ ID NO: 87 - RNA, 44 nt, synthetic construct
  misc_feature 1..44: note = Synthetic
  misc_feature 1: note = Polyethylene glycol (PEG) attached
  misc_feature 1..44: note = L-nucleic acid
  source 1..44: mol_type = other RNA
cggacacgcagctgtgggttgttgggaagtggtggtgtagtccg

SEQ ID NO: 88 - RNA, 40 nt, synthetic construct
  misc_feature 1..40: note = Synthetic
  misc_feature 1: note = Polyethylene glycol (PEG) attached
  misc_feature 1..40: note = L-nucleic acid
  misc_feature 3: note = Deoxyribonucleotide rather than ribonucleotide
  misc_feature 13: note = Deoxyribonucleotide rather than ribonucleotide
  misc_feature 34: note = Deoxyribonucleotide rather than ribonucleotide
  source 1..40: mol_type = other RNA
cgcacgcagctgtgggttgttgggaagtggtggtgtagcg

SEQ ID NO: 89 - protein, 74 aa, Mus musculus
  SITE 74: note = misc_feature - Biotin attached
LLRQKIEEQAAKYKHSVPKKCCYDGARVNFYETCEERVARVTIGPLCIRAFNECCTIANKIRKESPHKPVQLGR

SEQ ID NO: 90 - RNA, 44 nt, synthetic construct; identical to SEQ ID NO: 4
  misc_feature 1..44: note = Synthetic
  misc_feature 1: note = Polyethylene glycol (PEG) attached
  misc_feature 1..44: note = L-nucleic acid
  source 1..44: mol_type = other RNA

SEQ ID NO: 91 - RNA, 40 nt, synthetic construct; identical to SEQ ID NO: 37
  misc_feature 1..40: note = Synthetic
  misc_feature 1: note = Polyethylene glycol (PEG) attached
  misc_feature 1..40: note = L-nucleic acid
  misc_feature 7: note = Deoxyribonucleotide rather than ribonucleotide
  misc_feature 14: note = Deoxyribonucleotide rather than ribonucleotide
  misc_feature 15: note = Deoxyribonucleotide rather than ribonucleotide
  misc_feature 28: note = Deoxyribonucleotide rather than ribonucleotide
  misc_feature 30: note = Deoxyribonucleotide rather than ribonucleotide
  misc_feature 38: note = Deoxyribonucleotide rather than ribonucleotide
  source 1..40: mol_type = other RNA

SEQ ID NO: 92 - RNA, 40 nt, synthetic construct; identical to SEQ ID NO: 37
  misc_feature 1..40: note = Synthetic
  misc_feature 1: note = Polyethylene glycol (PEG) attached
  misc_feature 1..40: note = L-nucleic acid
  misc_feature 7: note = Deoxyribonucleotide rather than ribonucleotide
  misc_feature 28: note = Deoxyribonucleotide rather than ribonucleotide
  misc_feature 38: note = Deoxyribonucleotide rather than ribonucleotide
  source 1..40: mol_type = other RNA

SEQ ID NO: 93 - protein, 73 aa, Homo sapiens
TLQKKIEEIAAKYKHSVVKKCCYDGACVNNDETCEQRAARISLGPRCIKAFTECCVVASQLRANISHKDMQLG

SEQ ID NO: 94 - protein, 76 aa, Mus musculus
NLHLLRQKIEEQAAKYKHSVPKKCCYDGARVNFYETCEERVARVTIGPLCIRAFNECCTIANKIRKESPHKPVQLG

SEQ ID NO: 95 - DNA, 17 bp, synthetic construct
  source 1..17: mol_type = other DNA
  misc_feature 1: note = fluorescent dye Atto425 attached
  misc_feature 1..17: note = peptide nucleic acid
tgcgtcgacacccaaca